European Patent Specification EP 3 666 897 B1, published September 3, 2025. Title: A highly versatile method for presenting cyclic peptides on protein scaffolds. Applicant: The University of Tokyo Osaka University. The sequence listing filed with the application follows.

SEQUENCE LISTING (68 sequences)

SEQ ID NO: 1 - protein, 13 aa, Artificial Sequence
  variable region of cyclic peptide P6
RPRVARWTGQIIY

SEQ ID NO: 2 - protein, 13 aa, Artificial Sequence
  variable region of cyclic peptide mP6-9
RPYIERWTGRLIV

SEQ ID NO: 3 - protein, 13 aa, Artificial Sequence
  variable region of cyclic peptide P7
NSNVLSWQTYSWY

SEQ ID NO: 4 - protein, 14 aa, Artificial Sequence
  variable region of cyclic peptide aMD4
RQFNRRTHEVWNLD

SEQ ID NO: 5 - protein, 13 aa, Artificial Sequence
  variable region of cyclic peptide aMD5
WYYAWDQTYKAFP

SEQ ID NO: 6 - protein, 16 aa, Artificial Sequence
  variable region of cyclic peptide aML5
YISWNEFNSPNWRFIT

SEQ ID NO: 7 - protein, 15 aa, Artificial Sequence
  variable region of cyclic peptide A6-2f
ASFPEELDEWYVAYG

SEQ ID NO: 8 - protein, 11 aa, Artificial Sequence
  variable region of cyclic peptide trkD5
RQASPKFTFWS

SEQ ID NO: 9 - protein, 23 aa, Homo sapiens
TVYAVTGRGDSPASSKPISINYR

SEQ ID NO: 10 - protein, 35 aa, Artificial Sequence
  partial structure of Fn10(P6)-Fc
TVYAVTGRWRPRVARWTGQIIYSPASSKPISINYR

SEQ ID NO: 11 - protein, 35 aa, Artificial Sequence
  partial structure of Fn10(mP6-9)-Fc
TVYAVTGRWRPYIERWTGRLIVSPASSKPISINYR

SEQ ID NO: 12 - protein, 43 aa, Artificial Sequence
  partial structure of Fn10(P7)-Fc
TVYAVTGRGGSGCNSNVLSWQTYSWYCGGSSPASSKPISINYR

SEQ ID NO: 13 - protein, 39 aa, Artificial Sequence
  partial structure of Fn10(aMD4)-Fc
TVYAVTGRGGYRQFNRRTHEVWNLDGSPASSKPISINYR

SEQ ID NO: 14 - protein, 39 aa, Artificial Sequence
  partial structure of Fn10(aMD5)-Fc
TVYAVTGRGSYWYYAWDQTYKAFPGSSPASSKPISINYR

SEQ ID NO: 15 - protein, 40 aa, Artificial Sequence
  partial structure of Fn10(aML5)-Fc
TVYAVTGRGGYISWNEFNSPNWRFITGSPASSKPISINYR

SEQ ID NO: 16 - protein, 41 aa, Artificial Sequence
  partial structure of Fn10(A6-2f)-Fc
TVYAVTGRGGSYASFPEELDEWYVAYGGSPASSKPISINYR

SEQ ID NO: 17 - protein, 38 aa, Artificial Sequence
  partial structure of Fn10(trkD5)-Fc
TVYAVTGRGGSYRQASPKFTFWSGGSPASSKPISINYR

SEQ ID NO: 18 - protein, 14 aa, Homo sapiens
VVDVSHEDPEVKFN

SEQ ID NO: 19 - protein, 30 aa, Artificial Sequence
  partial structure of Fc(mP6-9_L1)
VVDVSHGWRPYIERWTGRLIVGGDPEVKFN

SEQ ID NO: 20 - protein, 32 aa, Artificial Sequence
  partial structure of Fc(aMD4_L1)
VVDVSHGGYRQFNRRTHEVWNLDGGDPEVKFN

SEQ ID NO: 21 - protein, 31 aa, Artificial Sequence
  partial structure of Fc(aMD5_L1)
VVDVSHGSYWYYAWDQTYKAFPGSDPEVKFN

SEQ ID NO: 22 - protein, 12 aa, Homo sapiens
REEQYNSTYRVV

SEQ ID NO: 23 - protein, 28 aa, Artificial Sequence
  partial structure of Fc(mP6-9_L2)
REEQYGWRPYIERWTGRLIVGNSTYRVV

SEQ ID NO: 24 - protein, 31 aa, Artificial Sequence
  partial structure of Fc(aMD4_L2)
REEQYGGYRQFNRRTHEVWNLDGSNSTYRVV

SEQ ID NO: 25 - protein, 30 aa, Artificial Sequence
  partial structure of Fc(aMD5_L2)
REEQYGSYWYYAWDQTYKAFPGSNSTYRVV

SEQ ID NO: 26 - protein, 13 aa, Homo sapiens
SNKALPAPIEKTI

SEQ ID NO: 27 - protein, 28 aa, Artificial Sequence
  partial structure of Fc(mP6-9_L3)
SNKALPGWRPYIERWTGRLIVGPIEKTI

SEQ ID NO: 28 - protein, 31 aa, Artificial Sequence
  partial structure of Fc(aMD4_L3)
SNKALPGGYRQFNRRTHEVWNLDGSPIEKTI

SEQ ID NO: 29 - protein, 30 aa, Artificial Sequence
  partial structure of Fc(aMD5_L3)
SNKALPGSYWYYAWDQTYKAFPGSPIEKTI

SEQ ID NO: 30 - protein, 12 aa, Homo sapiens
DELTKNQVSLTC

SEQ ID NO: 31 - protein, 28 aa, Artificial Sequence
  partial structure of Fc(mP6-9_L4)
DELTKGWRPYIERWTGRLIVGGQVSLTC

SEQ ID NO: 32 - protein, 30 aa, Artificial Sequence
  partial structure of Fc(aMD4_L4)
DELTKGGYRQFNRRTHEVWNLDGGQVSLTC

SEQ ID NO: 33 - protein, 31 aa, Artificial Sequence
  partial structure of Fc(aMD5_L4)
DELTKSGGYWYYAWDQTYKAFPGGSQVSLTC

SEQ ID NO: 34 - protein, 13 aa, Homo sapiens
VEWESNGQPENNY

SEQ ID NO: 35 - protein, 29 aa, Artificial Sequence
  partial structure of Fc(mP6-9_L5)
VEWESGWRPYIERWTGRLIVGGGQPENNY

SEQ ID NO: 36 - protein, 31 aa, Artificial Sequence
  partial structure of Fc(aMD4_L5)
VEWESGGYRQFNRRTHEVWNLDGGGQPENNY

SEQ ID NO: 37 - protein, 32 aa, Artificial Sequence
  partial structure of Fc(aMD5_L5)
VEWESSGGYWYYAWDQTYKAFPGGSGQPENNY

SEQ ID NO: 38 - protein, 12 aa, Homo sapiens
SRWQQGNVFSCS

SEQ ID NO: 39 - protein, 28 aa, Artificial Sequence
  partial structure of Fc(mP6-9_L6)
SRWQQGWRPYIERWTGRLIVGGNVFSCS

SEQ ID NO: 40 - protein, 30 aa, Artificial Sequence
  partial structure of Fc(aMD4_L6)
SRWQQGGYRQFNRRTHEVWNLDGGNVFSCS

SEQ ID NO: 41 - protein, 31 aa, Artificial Sequence
  partial structure of Fc(aMD5_L6)
SRWQQGSGYWYYAWDQTYKAFPGSGNVFSCS

SEQ ID NO: 42 - protein, 12 aa, Homo sapiens
SKSKGQPREPQV

SEQ ID NO: 43 - protein, 28 aa, Artificial Sequence
  partial structure of Fc(mP6-9_L7)
SKSKGWRPYIERWTGRLIVGGQPREPQV

SEQ ID NO: 44 - protein, 12 aa, Homo sapiens
PVLDSDGSFFLY

SEQ ID NO: 45 - protein, 28 aa, Artificial Sequence
  partial structure of Fc(mP6-9_L8)
PVLDSGWRPYIERWTGRLIVGGGSFFLY

SEQ ID NO: 46 - protein, 13 aa, Homo sapiens
TCVADESAENCDK

SEQ ID NO: 47 - protein, 29 aa, Artificial Sequence
  partial structure of HSA(mP6-9_L1)
TCVADEGWRPYIERWTGRLIVGGAENCDK

SEQ ID NO: 48 - protein, 31 aa, Artificial Sequence
  partial structure of HSA(aMD4_L1)
TCVADESGYRQFNRRTHEVWNLDGSAENCDK

SEQ ID NO: 49 - protein, 15 aa, Homo sapiens
FTECCQAADKAACLL

SEQ ID NO: 50 - protein, 31 aa, Artificial Sequence
  partial structure of HSA(mP6-9_L2)
FTECCQAGWRPYIERWTGRLIVGGDKAACLL

SEQ ID NO: 51 - protein, 33 aa, Artificial Sequence
  partial structure of HSA(aMD4_L2)
FTECCQAAGYRQFNRRTHEVWNLDGSDKAACLL

SEQ ID NO: 52 - protein, 14 aa, Homo sapiens
EKCCAAADPHECYA

SEQ ID NO: 53 - protein, 30 aa, Artificial Sequence
  partial structure of HSA(mP6-9_L3)
EKCCAAGWRPYIERWTGRLIVGGDPHECYA

SEQ ID NO: 54 - protein, 32 aa, Artificial Sequence
  partial structure of HSA(aMD4_L3)
EKCCAAAGYRQFNRRTHEVWNLDGSDPHECYA

SEQ ID NO: 55 - protein, 13 aa, Homo sapiens
KCCKADDKETCFA

SEQ ID NO: 56 - protein, 29 aa, Artificial Sequence
  partial structure of HSA(mP6-9_L4)
KCCKAGWRPYIERWTGRLIVGGDKETCFA

SEQ ID NO: 57 - protein, 31 aa, Artificial Sequence
  partial structure of HSA(aMD4_L4)
KCCKAGGYRQFNRRTHEVWNLDGGDKETCFA

SEQ ID NO: 58 - protein, 13 aa, Homo sapiens
MGRLEDGSPRTQA

SEQ ID NO: 59 - protein, 28 aa, Artificial Sequence
  partial structure of hGH(mP6-9_L1)
MGRLEDGWRPYIERWTGRLIVGSPRTQA

SEQ ID NO: 60 - protein, 14 aa, Homo sapiens
DANSHNDDALLKNY

SEQ ID NO: 61 - protein, 29 aa, Artificial Sequence
  partial structure of hGH(mP6-9_L2)
DANSHNGWRPYIERWTGRLIVGDALLKNY

SEQ ID NO: 62 - protein, 14 aa, Homo sapiens
GRVRLLNNWDVCAD

SEQ ID NO: 63 - protein, 30 aa, Artificial Sequence
  partial structure of RBP(mP6-9_L1)
GRVRLLGWRPYIERWTGRLIVGNNWDVCAD

SEQ ID NO: 64 - protein, 15 aa, Homo sapiens
KYWGVASFLQKGNDD

SEQ ID NO: 65 - protein, 31 aa, Artificial Sequence
  partial structure of RBP(mP6-9_L2)
KYWGVAGWRPYIERWTGRLIVGSFLQKGNDD

SEQ ID NO: 66 - protein, 14 aa, Homo sapiens
PGYVLKDGARPDVT

SEQ ID NO: 67 - protein, 32 aa, Artificial Sequence
  partial structure of PLAP(mP6-9)
PGYVLKGGWRPYIERWTGRLIVGGDGARPDVT

SEQ ID NO: 68 - protein, 33 aa, Artificial Sequence
  partial structure of PLAP(aMD4)
PGYVLKGGYRQFNRRTHEVWNLDGGDGARPDVT